European Patent Application EP 4 640 846 A1, published October 29, 2025. Title: A method for amplificating DNA using PCR. Applicant: ペプチドリーム株式会社. Application JP. The sequence listing filed with the application follows.

SEQUENCE LISTING (3 sequences)

SEQ ID NO: 1 - DNA, 106 bp, Synthetic construct
  source 1..106: mol_type = other DNA
ggcgtaatacgactcactataggtggggttcccgagcggccaaagggagcagactgtaaatctgccgtcacagacttcgaaggttcgaatccttcccccaccacca

SEQ ID NO: 2 - DNA, 23 bp, synthetic construct
  source 1..23: mol_type = other DNA
ccgcgtaatacgactcactatag

SEQ ID NO: 3 - DNA, 21 bp, Synthetic construct
  source 1..21: mol_type = other DNA
  modified_base 2: mod_base = OTHER; note = 2'-methylation
tggtggtgggggaaggattcg